European Patent Application EP 4 703 385 A1, published March 4, 2026. Title: 抗CD40L抗体及其在人自身免疫疾病治疗的应用. Applicant: 信达生物制药(苏州)有限公司. The sequence listing filed with the application follows.

SEQUENCE LISTING (32 sequences)

SEQ ID NO: 1 - protein, 10 aa, artificial sequence
GFTFSDYYMY

SEQ ID NO: 2 - protein, 17 aa, artificial sequence
TISGGGTYTYSPDSVKG

SEQ ID NO: 3 - protein, 7 aa, artificial sequence
GEPGLAY

SEQ ID NO: 4 - protein, 116 aa, artificial sequence
QVQLVESGGGLVKPGGSLRLSCAASGFTFSDYYMYWIRQAPGKGLEWVSTISGGGTYTYSPDSVKGRFTISRDNAKNSLYLQMNSLRAEDTAVYYCARGEPGLAYWGQGTLVTVSS

SEQ ID NO: 5 - protein, 329 aa, artificial sequence
ASTKGPSVFPLAPSSKSTSGGTAALGCLVKDYFPEPVTVSWNSGALTSGVHTFPAVLQSSGLYSLSSVVTVPSSSLGTQTYICNVNHKPSNTKVDKKVEPKSCDKTHTCPPCPAPEAAGGPSVFLFPPKPKDTLMISRTPEVTCVVVDVSHEDPEVKFNWYVDGVEVHNAKTKPREEQYNSTYRVVSVLTVLHQDWLNGKEYKCKVSNKALAPIEKTISKAKGQPREPQVYTLPPSRDELTKNQVSLTCLVKGFYPSDIAVEWESNGQPENNYKTTPPVLDSDGSFFLYSKLTVDKSRWQQGNVFSCSVMHEALHNHYTQKSLSLSPGK

SEQ ID NO: 6 - protein, 445 aa, artificial sequence
QVQLVESGGGLVKPGGSLRLSCAASGFTFSDYYMYWIRQAPGKGLEWVSTISGGGTYTYSPDSVKGRFTISRDNAKNSLYLQMNSLRAEDTAVYYCARGEPGLAYWGQGTLVTVSSASTKGPSVFPLAPSSKSTSGGTAALGCLVKDYFPEPVTVSWNSGALTSGVHTFPAVLQSSGLYSLSSVVTVPSSSLGTQTYICNVNHKPSNTKVDKKVEPKSCDKTHTCPPCPAPEAAGGPSVFLFPPKPKDTLMISRTPEVTCVVVDVSHEDPEVKFNWYVDGVEVHNAKTKPREEQYNSTYRVVSVLTVLHQDWLNGKEYKCKVSNKALAPIEKTISKAKGQPREPQVYTLPPSRDELTKNQVSLTCLVKGFYPSDIAVEWESNGQPENNYKTTPPVLDSDGSFFLYSKLTVDKSRWQQGNVFSCSVMHEALHNHYTQKSLSLSPGK

SEQ ID NO: 7 - protein, 15 aa, artificial sequence
KASQSVDYYGDSYMH

SEQ ID NO: 8 - protein, 7 aa, artificial sequence
ASSNLES

SEQ ID NO: 9 - protein, 9 aa, artificial sequence
QQSHEDPWT

SEQ ID NO: 10 - protein, 111 aa, artificial sequence
DIVMTQSPDSLAVSLGERATINCKASQSVDYYGDSYMHWYQQKPGQPPKLLIYASSNLESGVPDRFSGSGSGTDFTLTISSLQAEDVAVYYCQQSHEDPWTFGGGTKVEIK

SEQ ID NO: 11 - protein, 107 aa, artificial sequence [sequence omitted]

SEQ ID NO: 12 - protein, 218 aa, artificial sequence
DIVMTQSPDSLAVSLGERATINCKASQSVDYYGDSYMHWYQQKPGQPPKLLIYASSNLESGVPDRFSGSGSGTDFTLTISSLQAEDVAVYYCQQSHEDPWTFGGGTKVEIKRTVAAPSVFIFPPSDEQLKSGTASVVCLLNNFYPREAKVQWKVDNALQSGNSQESVTEQDSKDSTYSLSSTLTLSKADYEKHKVYACEVTHQGLSSPVTKSFNRGEC

SEQ ID NO: 13 - protein, 10 aa, artificial sequence
GFTFSDYAMS

SEQ ID NO: 14 - protein, 17 aa, artificial sequence
EISTVHTYTYYSDAVAG

SEQ ID NO: 15 - protein, 6 aa, artificial sequence
DRVLDY

SEQ ID NO: 16 - protein, 115 aa, artificial sequence
EVQLVESGGGLVKPGGSLRLSCAASGFTFSDYAMSWVRQAPGKGLEWVSEISTVHTYTYYSDAVAGRFTISRDNAKNSLYLQMNSLRAEDTAVYYCARDRVLDYWGQGTLVTVSS

SEQ ID NO: 17 - protein, 444 aa, artificial sequence
EVQLVESGGGLVKPGGSLRLSCAASGFTFSDYAMSWVRQAPGKGLEWVSEISTVHTYTYYSDAVAGRFTISRDNAKNSLYLQMNSLRAEDTAVYYCARDRVLDYWGQGTLVTVSSASTKGPSVFPLAPSSKSTSGGTAALGCLVKDYFPEPVTVSWNSGALTSGVHTFPAVLQSSGLYSLSSVVTVPSSSLGTQTYICNVNHKPSNTKVDKKVEPKSCDKTHTCPPCPAPEAAGGPSVFLFPPKPKDTLMISRTPEVTCVVVDVSHEDPEVKFNWYVDGVEVHNAKTKPREEQYNSTYRVVSVLTVLHQDWLNGKEYKCKVSNKALAPIEKTISKAKGQPREPQVYTLPPSRDELTKNQVSLTCLVKGFYPSDIAVEWESNGQPENNYKTTPPVLDSDGSFFLYSKLTVDKSRWQQGNVFSCSVMHEALHNHYTQKSLSLSPGK

SEQ ID NO: 18 - protein, 15 aa, artificial sequence
RASESVEYYDTSLMQ

SEQ ID NO: 19 - protein, 7 aa, artificial sequence
AASNLES

SEQ ID NO: 20 - protein, 9 aa, artificial sequence
QQTKKLPWT

SEQ ID NO: 21 - protein, 111 aa, artificial sequence
DIVMTQSPDSLAVSLGERATINCRASESVEYYDTSLMQWYQQKPGQPPKLLIYAASNLESGVPDRFSGSGSGTDFTLTISSLQAEDVAVYYCQQTKKLPWTFGQGTKVEIK

SEQ ID NO: 22 - protein, 218 aa, artificial sequence
DIVMTQSPDSLAVSLGERATINCRASESVEYYDTSLMQWYQQKPGQPPKLLIYAASNLESGVPDRFSGSGSGTDFTLTISSLQAEDVAVYYCQQTKKLPWTFGQGTKVEIKRTVAAPSVFIFPPSDEQLKSGTASVVCLLNNFYPREAKVQWKVDNALQSGNSQESVTEQDSKDSTYSLSSTLTLSKADYEKHKVYACEVTHQGLSSPVTKSFNRGEC

SEQ ID NO: 23 - protein, 227 aa, artificial sequence
DKTHTCPPCPAPELLGGPSVFLFPPKPKDTLMISRTPEVTCVVVDVSHEDPEVKFNWYVDGVEVHNAKTKPREEQYNSTYRVVSVLTVLHQDWLNGKEYKCKVSNKALPAPIEKTISKAKGQPREPQVYTLPPSRDELTKNQVSLTCLVKGFYPSDIAVEWESNGQPENNYKTTPPVLDSDGSFFLYSKLTVDKSRWQQGNVFSCSVMHEALHNHYTQKSLSLSPGK

SEQ ID NO: 24 - protein, 226 aa, artificial sequence
DKTHTCPPCPAPEAAGGPSVFLFPPKPKDTLMISRTPEVTCVVVDVSHEDPEVKFNWYVDGVEVHNAKTKPREEQYNSTYRVVSVLTVLHQDWLNGKEYKCKVSNKALAPIEKTISKAKGQPREPQVYTLPPSRDELTKNQVSLTCLVKGFYPSDIAVEWESNGQPENNYKTTPPVLDSDGSFFLYSKLTVDKSRWQQGNVFSCSVMHEALHNHYTQKSLSLSPGK

SEQ ID NO: 25 - protein, 103 aa, artificial sequence
ASTKGPSVFPLAPSSKSTSGGTAALGCLVKDYFPEPVTVSWNSGALTSGVHTFPAVLQSSGLYSLSSVVTVPSSSLGTQTYICNVNHKPSNTKVDKKVEPKSC

SEQ ID NO: 26 - protein, 330 aa, artificial sequence [sequence omitted]

SEQ ID NO: 27 - protein, 261 aa, artificial sequence
MIETYNQTSPRSAATGLPISMKIFMYLLTVFLITQMIGSALFAVYLHRRLDKIEDERNLHEDFVFMKTIQRCNTGERSLSLLNCEEIKSQFEGFVKDIMLNKEETKKENSFEMQKGDQNPQIAAHVISEASSKTTSVLQWAEKGYYTMSNNLVTLENGKQLTVKRQGLYYIYAQVTFCSNREASSQAPFIASLCLKSPGRFERILLRAANTHSSAKPCGQQSIHLGGVFELQPGASVFVNVTDPSQVSHGTGFTSFGLLKL

SEQ ID NO: 28 - protein, 1419 aa, artificial sequence
AAGCTTGCCGCCACCATGAAGTGGGTGACTTTTATCAGTCTACTATTCCTGTTCTCCTCCAGCTCTCGGGCTCAAGTGCAGCTGGTCGAGTCTGGCGGAGGCCTGGTGAAGCCTGGAGGCTCTCTCCGGCTGTCCTGTGCAGCCTCTGGCTTCACCTTCTCTGACTACTACATGTACTGGATCAGACAGGCCCCTGGCAAGGGACTGGAATGGGTGTCAACAATCAGCGGCGGCGGAACCTACACCTATTCTCCTGATTCCGTCAAGGGCAGATTCACCATCAGCCGGGACAACGCCAAGAACTCCCTGTACCTGCAGATGAACTCCCTGAGAGCCGAGGATACCGCCGTGTACTACTGCGCCAGAGGCGAGCCTGGCCTGGCCTACTGGGGACAAGGGACCCTCGTGACCGTGTCGTCCGCCTCCACCAAGGGACCTTCTGTGTTTCCTCTGGCTCCTAGCTCCAAGTCCACCTCCGGCGGCACCGCTGCTCTGGGCTGTCTGGTGAAGGACTACTTCCCTGAGCCCGTGACAGTGTCCTGGAACTCTGGCGCCCTGACCAGCGGCGTGCATACCTTTCCCGCTGTGTTGCAGTCCTCTGGCCTGTACTCTCTGTCTTCCGTGGTCACCGTGCCTTCATCCTCCCTGGGCACCCAGACCTACATCTGCAACGTGAACCACAAGCCCTCCAACACCAAGGTGGACAAGAAAGTGGAACCCAAATCTTGCGACAAGACCCACACCTGTCCTCCTTGCCCTGCTCCCGAGGCCGCTGGCGGCCCTTCCGTCTTTCTGTTCCCACCTAAGCCTAAGGATACACTGATGATCTCTAGAACACCTGAAGTGACCTGCGTGGTGGTCGACGTGTCTCACGAGGATCCAGAGGTGAAGTTCAATTGGTACGTGGATGGCGTGGAAGTGCACAACGCCAAAACCAAACCTAGAGAGGAACAGTACAACTCCACCTACAGAGTGGTTTCTGTCCTGACCGTGCTGCACCAGGACTGGCTGAACGGCAAAGAGTACAAGTGCAAGGTGAGCAACAAGGCCCTGGCCCCTATCGAGAAGACCATCTCCAAGGCTAAGGGCCAGCCCCGGGAACCTCAGGTTTATACACTGCCCCCATCTCGGGACGAGCTGACCAAGAACCAGGTGTCTCTGACCTGCCTGGTGAAAGGCTTCTACCCCTCTGACATCGCCGTGGAATGGGAGTCCAATGGCCAGCCTGAGAACAACTACAAGACAACCCCTCCTGTGCTGGACTCCGACGGCTCCTTCTTCCTGTACTCCAAGCTGACAGTGGACAAGTCCCGCTGGCAGCAGGGCAACGTGTTCTCCTGCTCCGTGATGCACGAGGCTCTGCATAATCACTACACCCAGAAGAGCCTGTCACTGTCTCCAGGCAAGTGATGAGAATTC

SEQ ID NO: 29 - protein, 738 aa, artificial sequence
AAGCTTGCCGCCACCATGAAGTGGGTGACTTTTATCAGTCTACTATTTCTGTTCTCCTCCAGCTCTAGAGCCGACATCGTGATGACCCAGAGTCCCGATAGCCTGGCTGTGTCCCTGGGAGAGCGCGCTACCATCAACTGCAAAGCCTCTCAGTCCGTGGATTACTACGGCGACTCCTACATGCACTGGTACCAGCAGAAGCCTGGCCAGCCTCCTAAGCTGCTGATCTACGCCTCTTCCAACCTGGAATCCGGCGTGCCCGACCGGTTTAGCGGCTCCGGCTCTGGTACCGACTTCACCCTCACAATCAGCTCTCTGCAGGCCGAGGACGTGGCCGTGTACTACTGCCAGCAGTCTCACGAGGATCCTTGGACCTTCGGCGGCGGAACAAAAGTGGAAATCAAGCGGACCGTGGCTGCTCCTTCCGTGTTCATCTTCCCCCCATCTGATGAACAGCTGAAGAGCGGCACAGCTTCTGTGGTGTGCCTGCTGAACAACTTCTACCCTAGAGAGGCCAAGGTGCAGTGGAAGGTGGACAACGCCCTGCAATCTGGCAACTCCCAAGAGTCCGTCACCGAGCAGGACTCCAAGGACTCTACCTACTCCCTGTCCTCCACCCTGACCCTGTCCAAAGCTGACTACGAGAAGCACAAGGTCTATGCCTGCGAGGTGACCCATCAGGGCCTGTCTTCTCCTGTGACCAAGTCCTTCAATAGAGGCGAATGTTGATGAGAATTC

SEQ ID NO: 30 - protein, 1416 aa, artificial sequence
AAGCTTGCCGCCACCATGAAGTGGGTGACTTTTATCAGTCTACTATTTCTGTTCTCCTCTTCCTCTAGAGCCGAGGTGCAGCTGGTGGAATCCGGCGGAGGCCTGGTCAAGCCTGGAGGCTCTCTGAGACTGTCCTGTGCCGCTTCCGGCTTCACCTTCAGCGACTACGCCATGTCTTGGGTGCGGCAGGCCCCTGGCAAGGGCCTGGAATGGGTCTCTGAGATCAGCACCGTGCACACCTATACCTATTACAGCGACGCCGTGGCCGGCAGATTCACCATCTCTCGGGACAACGCTAAGAACAGCCTGTACCTGCAGATGAACTCCCTCCGGGCTGAGGACACCGCCGTGTACTACTGCGCCAGAGATCGGGTGCTGGATTACTGGGGCCAAGGCACCCTGGTTACAGTCTCCTCCGCCTCTACCAAGGGACCAAGCGTGTTTCCTCTGGCCCCGAGTTCTAAGTCCACCTCTGGCGGCACCGCTGCCCTGGGCTGCCTGGTGAAGGACTACTTCCCTGAGCCCGTGACCGTGTCCTGGAACTCTGGCGCTCTGACCTCTGGTGTGCATACTTTCCCCGCTGTGCTGCAGTCCTCTGGACTGTACTCCCTGTCTTCGGTCGTGACAGTGCCCTCTAGCTCTCTGGGCACACAGACCTACATCTGCAACGTGAATCACAAGCCCTCCAACACCAAGGTGGACAAGAAAGTGGAACCTAAGTCTTGCGACAAGACACACACCTGTCCTCCTTGCCCTGCTCCTGAGGCTGCTGGCGGCCCTTCCGTGTTCCTGTTTCCACCCAAGCCTAAAGATACCCTGATGATCTCCCGGACCCCTGAAGTGACCTGCGTGGTGGTGGACGTGTCTCACGAAGATCCTGAAGTGAAGTTCAACTGGTACGTGGACGGCGTGGAAGTGCACAACGCCAAAACCAAACCTCGCGAAGAGCAGTACAACTCCACCTACAGAGTGGTCTCCGTGCTGACCGTGCTGCACCAGGACTGGCTGAACGGCAAAGAGTACAAGTGCAAGGTTTCCAACAAGGCTCTGGCTCCCATCGAGAAGACCATCTCCAAGGCCAAAGGCCAGCCTAGAGAGCCTCAGGTGTACACACTGCCTCCTAGCAGAGACGAGCTGACAAAGAACCAGGTGTCTTTGACCTGTCTGGTGAAGGGCTTCTACCCTTCTGACATCGCCGTGGAGTGGGAGTCCAATGGCCAACCCGAGAACAACTACAAGACCACCCCACCTGTGCTGGACTCCGATGGCTCCTTCTTCCTGTACTCCAAGCTGACCGTGGATAAGTCCAGATGGCAGCAGGGCAACGTGTTCTCCTGCTCTGTGATGCACGAGGCCCTGCATAATCACTACACCCAGAAGTCCCTGTCCCTAAGCCCTGGTAAGTGATGAGAATTC

SEQ ID NO: 31 - protein, 738 aa, artificial sequence
AAGCTTGCCGCCACCATGAAGTGGGTGACTTTTATCAGTCTACTATTTCTGTTCTCCAGCTCTTCTCGGGCCGATATCGTGATGACCCAGTCTCCAGATTCTCTGGCTGTGTCCCTGGGCGAAAGAGCTACCATCAACTGCAGAGCCTCCGAGTCCGTGGAATACTACGACACCAGCCTGATGCAGTGGTACCAGCAGAAGCCTGGCCAGCCTCCTAAGCTGCTGATCTACGCCGCTTCCAACCTGGAATCCGGCGTGCCCGACCGGTTTAGCGGATCTGGCTCTGGCACCGACTTCACCCTGACCATCTCCTCTCTCCAGGCCGAGGACGTGGCCGTGTACTACTGCCAGCAGACCAAGAAGCTGCCTTGGACCTTCGGCCAAGGCACCAAAGTCGAGATCAAGCGGACCGTGGCTGCTCCTTCCGTGTTCATCTTCCCCCCCTCCGATGAACAGCTGAAGTCTGGCACAGCTTCTGTGGTGTGCCTGCTGAACAACTTCTACCCTAGAGAGGCCAAAGTGCAGTGGAAGGTGGACAATGCCCTGCAGTCCGGCAACTCCCAAGAGTCTGTTACTGAGCAGGACTCCAAGGACTCTACCTACTCCCTGAGCTCCACCCTGACACTGTCTAAGGCCGACTACGAGAAGCACAAAGTCTATGCCTGCGAGGTGACACACCAGGGACTGTCCAGCCCTGTGACCAAGTCCTTCAACAGAGGCGAGTGTTGATGAGAATTC

SEQ ID NO: 32 - protein, 257 aa, artificial sequence
EPPTACREKQYLINSQCCSLCQPGQKLVSDCTEFTETECLPCGESEFLDTWNRETHCHQHKYCDPNLGLRVQQKGTSETDTICTCEEGWHCTSEACESCVLHRSCSPGFGVKQIATGVSDTICEPCPVGFFSNVSSAFEKCHPWTSCETKDLVVQQAGTNKTDVVCGPQDRLRALVVIPIIFGILFAILLVLVFIKKVAKKPTNKAPHPKQEPQEINFPDDLPGSNTAAPVQETLHGCQPVTQEDGKESRISVQERQ